European Patent Specification EP 3 833 690 B1, published March 27, 2024. Title: RECOMBINANT BIFUNCTIONAL PROTEIN TARGETING CD47 AND HER2. Applicant: ImmuneOnco BioPharmaceuticals (Shanghai) Co., Ltd. The sequence listing filed with the application follows.

SEQUENCE LISTING (20 sequences)

SEQ ID NO: 1 - DNA, 375 bp, Artificial Sequence
  Nucleotides encoding first extracellular Ig-like domain of SIRPalpha
gaggaggagctgcaggtgattcagcctgacaagtccgtatcagttgcagctggagagtcggccattctgcactgcactgtgacctccctgatccctgtggggcccatccagtggttcagaggagctggaccagcccgggaattaatctacaatcaaaaagaaggccacttcccccgggtaacaactgtttcagagtccacaaagagagaaaacatggacttttccatcagcatcagtgccatcaccccagcagatgccggcacctactactgtgtgaagttccggaaagggagccctgacacggagtttaagtctggagcaggcactgagctgtctgtgcgtgccaaaccctctgcccccgtggtatcgggccct

SEQ ID NO: 2 - protein, 125 aa, Homo sapiens
EEELQVIQPDKSVSVAAGESAILHCTVTSLIPVGPIQWFRGAGPARELIYNQKEGHFPRVTTVSESTKRENMDFSISISAITPADAGTYYCVKFRKGSPDTEFKSGAGTELSVRAKPSAPVVSGP

SEQ ID NO: 3 - DNA, 45 bp, Artificial Sequence
  Nucleotides encoding linker
ggcggcggtgggagcggcggcggtgggagcggcggcgggggctcg

SEQ ID NO: 4 - protein, 15 aa, Artificial Sequence
  Linker
GGGGSGGGGSGGGGS

SEQ ID NO: 5 - DNA, 1353 bp, Artificial Sequence
  Nucleotides encoding heavy chain of anti-HER2 antibody
gaggtgcagctggtcgagagcggcgggggcctcgtgcagccgggcgggtcgctgcggctgagctgcgccgcgagcgggttcaacatcaaggacacctacatccactgggtgcgccaggcccccggcaagggcctcgagtgggtcgcccggatctaccccacgaacgggtacacccgctacgccgacagcgtgaagggccggttcaccatcagcgcggacacctcgaagaacacggcctacctgcagatgaacagcctgcgcgccgaggacaccgccgtgtactactgcagccggtggggcggcgacgggttctacgccatggactactgggggcagggcaccctcgtcaccgtgagcagcgctagcaccaagggcccatcggtcttccccctggcaccctcctccaagagcacctctgggggcacagcggccctgggctgcctggtcaaggactacttccccgaaccggtgacggtgtcgtggaactcaggcgccctgaccagcggcgtgcacaccttcccggctgtcctacagtcctcaggactctactccctcagcagcgtggtgaccgtgccctccagcagcttgggcacccagacctacatctgcaacgtgaatcacaagcccagcaacaccaaggtggacaagagagttgagcccaaatcttgtgacaaaactcacacatgcccaccgtgcccagcacctgaactcctggggggaccgtcagtcttcctcttccccccaaaacccaaggacaccctcatgatctcccggacccctgaggtcacatgcgtggtggtggacgtgagccacgaagaccctgaggtcaagttcaactggtatgtggacggcgtggaggtgcataatgccaagacaaagccgcgggaggagcagtacaacgccacgtaccgtgtggtcagcgtcctcaccgtcctgcaccaagactggctgaatggcaaggagtacaagtgcaaggtctccaacaaagccctcccagcccccatcgccgcaaccatctccaaagccaaagggcagccccgagaaccacaggtgtacaccctgcccccatcccgggaggagatgaccaagaaccaagtcagcctgacctgcctggtcaaaggcttctatcccagcgacatcgccgtggagtgggagagcaatgggcagccggagaacaactacaagaccacgcctcccgtgctggactccgacggctccttcttcctctattccaagctcaccgtggacaagagcaggtggcagcaggggaacgtcttctcatgctccgtgatgcatgaggctctgcacaaccactacacgcagaagagcctctccctgtctccgggcaaatga

SEQ ID NO: 6 - protein, 450 aa, Artificial Sequence
  Heavy chain of anti-HER2 antibody
EVQLVESGGGLVQPGGSLRLSCAASGFNIKDTYIHWVRQAPGKGLEWVARIYPTNGYTRYADSVKGRFTISADTSKNTAYLQMNSLRAEDTAVYYCSRWGGDGFYAMDYWGQGTLVTVSSASTKGPSVFPLAPSSKSTSGGTAALGCLVKDYFPEPVTVSWNSGALTSGVHTFPAVLQSSGLYSLSSVVTVPSSSLGTQTYICNVNHKPSNTKVDKRVEPKSCDKTHTCPPCPAPELLGGPSVFLFPPKPKDTLMISRTPEVTCVVVDVSHEDPEVKFNWYVDGVEVHNAKTKPREEQYNATYRVVSVLTVLHQDWLNGKEYKCKVSNKALPAPIAATISKAKGQPREPQVYTLPPSREEMTKNQVSLTCLVKGFYPSDIAVEWESNGQPENNYKTTPPVLDSDGSFFLYSKLTVDKSRWQQGNVFSCSVMHEALHNHYTQKSLSLSPGK

SEQ ID NO: 7 - DNA, 645 bp, Artificial Sequence
  Nucleotides encoding light chain of anti-HER2 antibody
gacatccagatgacccagagcccgtcgagcctgagcgccagcgtgggcgaccgggtcacgatcacctgccgcgcgagccaggacgtgaacaccgccgtggcctggtaccagcagaagcccgggaaggcccccaagctcctgatctactcggcgagcttcctgtacagcggcgtccccagccggttcagcgggtcgcgcagcggcaccgacttcacgctcaccatcagcagcctgcagccggaggacttcgccacctactactgccagcagcactacaccacgccccccaccttcgggcagggcaccaaggtggagatcaagcgaactgtggctgcaccatctgtcttcatcttcccgccatctgatgagcagttgaaatctggaactgcctctgttgtgtgcctgctgaataacttctatcccagagaggccaaagtacagtggaaggtggataacgccctccaatcgggtaactcccaggagagtgtcacagagcaggacagcaaggacagcacctacagcctcagcagcaccctgacgctgagcaaagcagactacgagaaacacaaagtctacgcctgcgaagtcacccatcagggcctgagctcgcccgtcacaaagagcttcaacaggggagagtgttag

SEQ ID NO: 8 - protein, 214 aa, Artificial Sequence
  Light chain of anti-HER2 antibody
DIQMTQSPSSLSASVGDRVTITCRASQDVNTAVAWYQQKPGKAPKLLIYSASFLYSGVPSRFSGSRSGTDFTLTISSLQPEDFATYYCQQHYTTPPTFGQGTKVEIKRTVAAPSVFIFPPSDEQLKSGTASVVCLLNNFYPREAKVQWKVDNALQSGNSQESVTEQDSKDSTYSLSSTLTLSKADYEKHKVYACEVTHQGLSSPVTKSFNRGEC

SEQ ID NO: 9 - DNA, 1773 bp, Artificial Sequence
  Nucleotides encoding SIRP alpha D1-Linker-anti-HER2 heavy chain
gaggaggagctgcaggtgattcagcctgacaagtccgtatcagttgcagctggagagtcggccattctgcactgcactgtgacctccctgatccctgtggggcccatccagtggttcagaggagctggaccagcccgggaattaatctacaatcaaaaagaaggccacttcccccgggtaacaactgtttcagagtccacaaagagagaaaacatggacttttccatcagcatcagtgccatcaccccagcagatgccggcacctactactgtgtgaagttccggaaagggagccctgacacggagtttaagtctggagcaggcactgagctgtctgtgcgtgccaaaccctctgcccccgtggtatcgggccctggcggcggtgggagcggcggcggtgggagcggcggcgggggctcggaggtgcagctggtcgagagcggcgggggcctcgtgcagccgggcgggtcgctgcggctgagctgcgccgcgagcgggttcaacatcaaggacacctacatccactgggtgcgccaggcccccggcaagggcctcgagtgggtcgcccggatctaccccacgaacgggtacacccgctacgccgacagcgtgaagggccggttcaccatcagcgcggacacctcgaagaacacggcctacctgcagatgaacagcctgcgcgccgaggacaccgccgtgtactactgcagccggtggggcggcgacgggttctacgccatggactactgggggcagggcaccctcgtcaccgtgagcagcgctagcaccaagggcccatcggtcttccccctggcaccctcctccaagagcacctctgggggcacagcggccctgggctgcctggtcaaggactacttccccgaaccggtgacggtgtcgtggaactcaggcgccctgaccagcggcgtgcacaccttcccggctgtcctacagtcctcaggactctactccctcagcagcgtggtgaccgtgccctccagcagcttgggcacccagacctacatctgcaacgtgaatcacaagcccagcaacaccaaggtggacaagagagttgagcccaaatcttgtgacaaaactcacacatgcccaccgtgcccagcacctgaactcctggggggaccgtcagtcttcctcttccccccaaaacccaaggacaccctcatgatctcccggacccctgaggtcacatgcgtggtggtggacgtgagccacgaagaccctgaggtcaagttcaactggtatgtggacggcgtggaggtgcataatgccaagacaaagccgcgggaggagcagtacaacgccacgtaccgtgtggtcagcgtcctcaccgtcctgcaccaagactggctgaatggcaaggagtacaagtgcaaggtctccaacaaagccctcccagcccccatcgccgcaaccatctccaaagccaaagggcagccccgagaaccacaggtgtacaccctgcccccatcccgggaggagatgaccaagaaccaagtcagcctgacctgcctggtcaaaggcttctatcccagcgacatcgccgtggagtgggagagcaatgggcagccggagaacaactacaagaccacgcctcccgtgctggactccgacggctccttcttcctctattccaagctcaccgtggacaagagcaggtggcagcaggggaacgtcttctcatgctccgtgatgcatgaggctctgcacaaccactacacgcagaagagcctctccctgtctccgggcaaatga

SEQ ID NO: 10 - protein, 590 aa, Artificial Sequence
  SIRP alpha D1-Linker-anti-HER2 heavy chain
EEELQVIQPDKSVSVAAGESAILHCTVTSLIPVGPIQWFRGAGPARELIYNQKEGHFPRVTTVSESTKRENMDFSISISAITPADAGTYYCVKFRKGSPDTEFKSGAGTELSVRAKPSAPVVSGPGGGGSGGGGSGGGGSEVQLVESGGGLVQPGGSLRLSCAASGFNIKDTYIHWVRQAPGKGLEWVARIYPTNGYTRYADSVKGRFTISADTSKNTAYLQMNSLRAEDTAVYYCSRWGGDGFYAMDYWGQGTLVTVSSASTKGPSVFPLAPSSKSTSGGTAALGCLVKDYFPEPVTVSWNSGALTSGVHTFPAVLQSSGLYSLSSVVTVPSSSLGTQTYICNVNHKPSNTKVDKRVEPKSCDKTHTCPPCPAPELLGGPSVFLFPPKPKDTLMISRTPEVTCVVVDVSHEDPEVKFNWYVDGVEVHNAKTKPREEQYNATYRVVSVLTVLHQDWLNGKEYKCKVSNKALPAPIAATISKAKGQPREPQVYTLPPSREEMTKNQVSLTCLVKGFYPSDIAVEWESNGQPENNYKTTPPVLDSDGSFFLYSKLTVDKSRWQQGNVFSCSVMHEALHNHYTQKSLSLSPGK

SEQ ID NO: 11 - DNA, 1065 bp, Artificial Sequence
  Nucleotides encoding SIRP alpha D1-Linker-anti-HER2 light chain
gaggaggagctgcaggtgattcagcctgacaagtccgtatcagttgcagctggagagtcggccattctgcactgcactgtgacctccctgatccctgtggggcccatccagtggttcagaggagctggaccagcccgggaattaatctacaatcaaaaagaaggccacttcccccgggtaacaactgtttcagagtccacaaagagagaaaacatggacttttccatcagcatcagtgccatcaccccagcagatgccggcacctactactgtgtgaagttccggaaagggagccctgacacggagtttaagtctggagcaggcactgagctgtctgtgcgtgccaaaccctctgcccccgtggtatcgggccctggcggcggtgggagcggcggcggtgggagcggcggcgggggctcggacatccagatgacccagagcccgtcgagcctgagcgccagcgtgggcgaccgggtcacgatcacctgccgcgcgagccaggacgtgaacaccgccgtggcctggtaccagcagaagcccgggaaggcccccaagctcctgatctactcggcgagcttcctgtacagcggcgtccccagccggttcagcgggtcgcgcagcggcaccgacttcacgctcaccatcagcagcctgcagccggaggacttcgccacctactactgccagcagcactacaccacgccccccaccttcgggcagggcaccaaggtggagatcaagcgaactgtggctgcaccatctgtcttcatcttcccgccatctgatgagcagttgaaatctggaactgcctctgttgtgtgcctgctgaataacttctatcccagagaggccaaagtacagtggaaggtggataacgccctccaatcgggtaactcccaggagagtgtcacagagcaggacagcaaggacagcacctacagcctcagcagcaccctgacgctgagcaaagcagactacgagaaacacaaagtctacgcctgcgaagtcacccatcagggcctgagctcgcccgtcacaaagagcttcaacaggggagagtgttag

SEQ ID NO: 12 - protein, 354 aa, Artificial Sequence
  SIRP alpha D1-Linker-anti-HER2 light chain
EEELQVIQPDKSVSVAAGESAILHCTVTSLIPVGPIQWFRGAGPARELIYNQKEGHFPRVTTVSESTKRENMDFSISISAITPADAGTYYCVKFRKGSPDTEFKSGAGTELSVRAKPSAPVVSGPGGGGSGGGGSGGGGSDIQMTQSPSSLSASVGDRVTITCRASQDVNTAVAWYQQKPGKAPKLLIYSASFLYSGVPSRFSGSRSGTDFTLTISSLQPEDFATYYCQQHYTTPPTFGQGTKVEIKRTVAAPSVFIFPPSDEQLKSGTASVVCLLNNFYPREAKVQWKVDNALQSGNSQESVTEQDSKDSTYSLSSTLTLSKADYEKHKVYACEVTHQGLSSPVTKSFNRGEC

SEQ ID NO: 13 - DNA, 1101 bp, Artificial Sequence
  Nucleotides encoding SIRP alpha D1-Fc
gaggaggagctgcaggtgattcagcctgacaagtccgtatcagttgcagctggagagtcggccattctgcactgcactgtgacctccctgatccctgtggggcccatccagtggttcagaggagctggaccagcccgggaattaatctacaatcaaaaagaaggccacttcccccgggtaacaactgtttcagagtccacaaagagagaaaacatggacttttccatcagcatcagtgccatcaccccagcagatgccggcacctactactgtgtgaagttccggaaagggagccctgacacggagtttaagtctggagcaggcactgagctgtctgtgcgtgccaaaccctctgcccccgtggtatcgggccctgcggcgagggccacacctcagcacgaattcgagcccaaatcttgtgacaaaactcacacatgcccaccgtgcccagcacctgaactcctggggggaccgtcagtcttcctcttccccccaaaacccaaggacaccctcatgatctcccggacccctgaggtcacatgcgtggtggtggacgtgagccacgaagaccctgaggtcaagttcaactggtacgtggacggcgtggaggtgcataatgccaagacaaagccgcgggaggagcagtacaacagcacgtaccgtgtggtcagcgtcctcaccgtcctgcaccaggactggctgaatggcaaggagtacaagtgcaaggtctccaacaaagccctcccagcccccatcgagaaaaccatctccaaagccaaagggcagccccgagaaccacaggtgtacaccctgcccccatcccgggatgagctgaccaagaaccaggtcagcctgacctgcctggtcaaaggcttctatcccagcgacatcgccgtggagtgggagagcaatgggcagccggagaacaactacaagaccacgcctcccgtgctggactccgacggctccttcttcctctacagcaagctcaccgtggacaagagcaggtggcagcaggggaacgtcttctcatgctccgtgatgcatgaggctctgcacaaccactacacgcagaagagcctctccctgtctccgggttga

SEQ ID NO: 14 - protein, 366 aa, Artificial Sequence
  SIRP alpha D1-Fc
EEELQVIQPDKSVSVAAGESAILHCTVTSLIPVGPIQWFRGAGPARELIYNQKEGHFPRVTTVSESTKRENMDFSISISAITPADAGTYYCVKFRKGSPDTEFKSGAGTELSVRAKPSAPVVSGPAARATPQHEFEPKSCDKTHTCPPCPAPELLGGPSVFLFPPKPKDTLMISRTPEVTCVVVDVSHEDPEVKFNWYVDGVEVHNAKTKPREEQYNSTYRVVSVLTVLHQDWLNGKEYKCKVSNKALPAPIEKTISKAKGQPREPQVYTLPPSRDELTKNQVSLTCLVKGFYPSDIAVEWESNGQPENNYKTTPPVLDSDGSFFLYSKLTVDKSRWQQGNVFSCSVMHEALHNHYTQKSLSLSPG

SEQ ID NO: 15 - DNA, 1749 bp, Artificial Sequence
  Nulcoetides encoding SIRP alpha D1-Linker-anti-EGFR light chain
gaggaggagctgcaggtgattcagcctgacaagtccgtatcagttgcagctggagagtcggccattctgcactgcactgtgacctccctgatccctgtggggcccatccagtggttcagaggagctggaccagcccgggaattaatctacaatcaaaaagaaggccacttcccccgggtaacaactgtttcagagtccacaaagagagaaaacatggacttttccatcagcatcagtgccatcaccccagcagatgccggcacctactactgtgtgaagttccggaaagggagccctgacacggagtttaagtctggagcaggcactgagctgtctgtgcgtgccaaaccctctggcggcggtgggagcggcggcggtgggagcggcggcgggggctcgcaggtgcagctgaagcagtcaggacctggcctagtgcagccctcacagagcctgtccatcacctgcacagtctctggtttctcattaactaactatggtgtacactgggttcgccagtctccaggaaagggtctggagtggctgggagtgatatggagtggtggaaacacagactataatacacctttcacatccagactgagcatcaacaaggacaattccaagagccaagttttctttaaaatgaacagtctgcaatctcaggacacagccatatattactgtgccagagccctcacctactatgattacgagtttgcttactggggccaagggactctggtcactgtctctgcagctagcaccaagggcccatcggtcttccccctggcaccctcctccaagagcacctctgggggcacagcggccctgggctgcctggtcaaggactacttccccgaaccggtgacggtgtcgtggaactcaggcgccctgaccagcggcgtgcacaccttcccggctgtcctacagtcctcaggactctactccctcagcagcgtggtgaccgtgccctccagcagcttgggcacccagacctacatctgcaacgtgaatcacaagcccagcaacaccaaggtggacaagagagttgagcccaaatcttgtgacaaaactcacacatgcccaccgtgcccagcacctgaactcctggggggaccgtcagtcttcctcttccccccaaaacccaaggacaccctcatgatctcccggacccctgaggtcacatgcgtggtggtggacgtgagccacgaagaccctgaggtcaagttcaactggtatgtggacggcgtggaggtgcataatgccaagacaaagccgcgggaggagcagtacaacgccacgtaccgtgtggtcagcgtcctcaccgtcctgcaccaagactggctgaatggcaaggagtacaagtgcaaggtctccaacaaagccctcccagcccccatcgccgcaaccatctccaaagccaaagggcagccccgagaaccacaggtgtacaccctgcccccatcccgggaggagatgaccaagaaccaagtcagcctgacctgcctggtcaaaggcttctatcccagcgacatcgccgtggagtgggagagcaatgggcagccggagaacaactacaagaccacgcctcccgtgctggactccgacggctccttcttcctctattccaagctcaccgtggacaagagcaggtggcagcaggggaacgtcttctcatgctccgtgatgcatgaggctctgcacaaccactacacgcagaagagcctctccctgtctccgggcaaatga

SEQ ID NO: 16 - protein, 582 aa, Artificial Sequence
  SIRP alpha D1-Linker-anti-EGFR light chain
EEELQVIQPDKSVSVAAGESAILHCTVTSLIPVGPIQWFRGAGPARELIYNQKEGHFPRVTTVSESTKRENMDFSISISAITPADAGTYYCVKFRKGSPDTEFKSGAGTELSVRAKPSGGGGSGGGGSGGGGSQVQLKQSGPGLVQPSQSLSITCTVSGFSLTNYGVHWVRQSPGKGLEWLGVIWSGGNTDYNTPFTSRLSINKDNSKSQVFFKMNSLQSQDTAIYYCARALTYYDYEFAYWGQGTLVTVSAASTKGPSVFPLAPSSKSTSGGTAALGCLVKDYFPEPVTVSWNSGALTSGVHTFPAVLQSSGLYSLSSVVTVPSSSLGTQTYICNVNHKPSNTKVDKRVEPKSCDKTHTCPPCPAPELLGGPSVFLFPPKPKDTLMISRTPEVTCVVVDVSHEDPEVKFNWYVDGVEVHNAKTKPREEQYNATYRVVSVLTVLHQDWLNGKEYKCKVSNKALPAPIAATISKAKGQPREPQVYTLPPSREEMTKNQVSLTCLVKGFYPSDIAVEWESNGQPENNYKTTPPVLDSDGSFFLYSKLTVDKSRWQQGNVFSCSVMHEALHNHYTQKSLSLSPGK

SEQ ID NO: 17 - DNA, 645 bp, Artificial Sequence
  Nucleotides encoding Light chain of anti-EGFR antibody
gacatcttgctgactcagtctccagtcatcctgtctgtgagtccaggagaaagagtcagtttctcctgcagggccagtcagagtattggcacaaacatacactggtatcagcaaagaacaaatggttctccaaggcttctcataaagtatgcttctgagtctatctctgggatcccttccaggtttagtggcagtggatcagggacagattttactcttagcatcaacagtgtggagtctgaagatattgcagattattactgtcaacaaaataataactggccaaccacgttcggtgctgggaccaagctggagctgaaacgaactgtggctgcaccatctgtcttcatcttcccgccatctgatgagcagttgaaatctggaactgcctctgttgtgtgcctgctgaataacttctatcccagagaggccaaagtacagtggaaggtggataacgccctccaatcgggtaactcccaggagagtgtcacagagcaggacagcaaggacagcacctacagcctcagcagcaccctgacgctgagcaaagcagactacgagaaacacaaagtctacgcctgcgaagtcacccatcagggcctgagctcgcccgtcacaaagagcttcaacaggggagagtgttag

SEQ ID NO: 18 - protein, 214 aa, Artificial Sequence
  Light chain of anti-EGFR antibody
DILLTQSPVILSVSPGERVSFSCRASQSIGTNIHWYQQRTNGSPRLLIKYASESISGIPSRFSGSGSGTDFTLSINSVESEDIADYYCQQNNNWPTTFGAGTKLELKRTVAAPSVFIFPPSDEQLKSGTASVVCLLNNFYPREAKVQWKVDNALQSGNSQESVTEQDSKDSTYSLSSTLTLSKADYEKHKVYACEVTHQGLSSPVTKSFNRGEC

SEQ ID NO: 19 - DNA, 57 bp, Artificial Sequence
  Nucleotides encoding signal peptide
atgggatggtcatgtatcatcctttttctggtagcaactgcaactggagtacattca

SEQ ID NO: 20 - DNA, 9 bp, Artificial Sequence
  Kozak
gccgccacc